European Patent Application EP 4 792 888 A1, published August 19, 2026. Title: Novel darobactin derivatives characterized by high activity against gram-negative pathogens. Applicant: Justus-Liebig-Universität Giessen. Application EP. The sequence listing filed with the application follows.

SEQUENCE LISTING (3 sequences)

SEQ ID NO: 1 - protein, 7 aa, synthetic construct
WNWRKRF

SEQ ID NO: 2 - protein, 7 aa, synthetic construct
WNWRKTF

SEQ ID NO: 3 - protein, 7 aa, synthetic construct
WNWSKSF